European Patent Specification EP 3 740 222 B1, published June 28, 2023. Title: A modified rAAV capsid protein for gene therapy. Applicant: Arthrogen B.V. Universität Heidelberg. The sequence listing filed with the application follows.

SEQUENCE LISTING (27 sequences)

SEQ ID NO: 1 - protein, 745 aa, Artificial Sequence
  AAV1 with insert P4
MAADGYLPDWLEDNLSEGIREWWDLKPGAPKPKANQQKQDDGRGLVLPGYKYLGPFNGLDKGEPVNAADAAALEHDKAYDQQLKAGDNPYLRYNHADAEFQERLQEDTSFGGNLGRAVFQAKKRVLEPLGLVEEGAKTAPGKKRPVEQSPQEPDSSSGIGKTGQQPAKKRLNFGQTGDSESVPDPQPLGEPPATPAAVGPTTMASGGGAPMADNNEGADGVGNASGNWHCDSTWLGDRVITTSTRTWALPTYNNHLYKQISSASTGASNDNHYFGYSTPWGYFDFNRFHCHFSPRDWQRLINNNWGFRPKRLNFKLFNIQVKEVTTNDGVTTIANNLTSTVQVFSDSEYQLPYVLGSAHQGCLPPFPADVFMIPQYGYLTLNNGSQAVGRSSFYCLEYFPSQMLRTGNNFTFSYTFEEVPFHSSYAHSQSLDRLMNPLIDQYLYYLNRTQNQSGSAQNKDLLFSRGSPAGMSVQPKNWLPGPCYRQQRVSKTKTDNNNSNFTWTGASKYNLNGRESIINPGTAMASHKDDEDKFFPMSGVMIFGKESAGASNTALDNVMITDEEEIKATNPVATERFGTVAVNFQSSGQSGNDVRSANAQAAGDVHAMGALPGMVWQDRDVYLQGPIWAKIPHTDGHFHPSPLMGGFGLKNPPPQILIKNTPVPANPPAEFSATKFASFITQYSTGQVSVEIEWELQKENSKRWNPEVQYTSNYAKSANVDFTVDNNGLYTEPRPIGTRYLTRPL

SEQ ID NO: 2 - protein, 746 aa, Artificial Sequence
  AAV2 with insert P2
MAADGYLPDWLEDTLSEGIRQWWKLKPGPPPPKPAERHKDDSRGLVLPGYKYLGPFNGLDKGEPVNEADAAALEHDKAYDRQLDSGDNPYLKYNHADAEFQERLKEDTSFGGNLGRAVFQAKKRVLEPLGLVEEPVKTAPGKKRPVEHSPVEPDSSSGTGKAGQQPARKRLNFGQTGDADSVPDPQPLGQPPAAPSGLGTNTMATGSGAPMADNNEGADGVGNSSGNWHCDSTWMGDRVITTSTRTWALPTYNNHLYKQISSQSGASNDNHYFGYSTPWGYFDFNRFHCHFSPRDWQRLINNNWGFRPKRLNFKLFNIQVKEVTQNDGTTTIANNLTSTVQVFTDSEYQLPYVLGSAHQGCLPPFPADVFMVPQYGYLTLNNGSQAVGRSSFYCLEYFPSQMLRTGNNFTFSYTFEDVPFHSSYAHSQSLDRLMNPLIDQYLYYLSRTNTPSGTTTQSRLQFSQAGASDIRDQSRNWLPGPCYRQQRVSKTSADNNNSEYSWTGATKYHLNGRDSLVNPGPAMASHKDDEEKFFPQSGVLIFGKQGSEKTNVDIEKVMITDEEEIRTTNPVATEQYGSVSTNLQQGQSGCDCRGDCFCAQAATADVNTQGVLPGMVWQDRDVYLQGPIWAKIPHTDGHFHPSPLMGGFGLKHPPPQILIKNTPVPANPSTTFSAAKFASFITQYSTGQVSVEIEWELQKENSKRWNPEIQYTSNYNKSVNVDFTVDTNGVYSEPRPIGTRYLTRNL

SEQ ID NO: 3 - protein, 746 aa, Artificial Sequence
  AAV7 with insert A6
MAADGYLPDWLEDNLSEGIREWWDLKPGAPKPKANQQKQDNGRGLVLPGYKYLGPFNGLDKGEPVNAADAAALEHDKAYDQQLKAGDNPYLRYNHADAEFQERLQEDTSFGGNLGRAVFQAKKRVLEPLGLVEEGAKTAPAKKRPVEPSPQRSPDSSTGIGKKGQQPARKRLNFGQTGDSESVPDPQPLGEPPAAPSSVGSGTVAAGGGAPMADNNEGADGVGNASGNWHCDSTWLGDRVITTSTRTWALPTYNNHLYKQISSETAGSTNDNTYFGYSTPWGYFDFNRFHCHFSPRDWQRLINNNWGFRPKKLRFKLFNIQVKEVTTNDGVTTIANNLTSTIQVFSDSEYQLPYVLGSAHQGCLPPFPADVFMIPQYGYLTLNNGSQSVGRSSFYCLEYFPSQMLRTGNNFEFSYSFEDVPFHSSYAHSQSLDRLMNPLIDQYLYYLARTQSNPGGTAGNRELQFYQGGPSTMAEQAKNWLPGPCFRQQRVSKTLDQNNNSNFAWTGATKYHLNGRNSLVNPGVAMATHKDDEDRFFPSSGVLIFGKTGATNKTTLENVLMTNEEEIRPTNPVATEEYGIVSSNLQGQRGNEARVREAQAAQTQVVNNQGALPGMVWQNRDVYLQGPIWAKIPHTDGNFHPSPLMGGFGLKHPPPQILIKNTPVPANPPEVFTPAKFASFITQYSTGQVSVEIEWELQKENSKRWNPEIQYTSNFEKQTGVDFAVDSQGVYSEPRPIGTRYLTRNL

SEQ ID NO: 4 - protein, 745 aa, Artificial Sequence
  AAV9 with insert A2
MAADGYLPDWLEDNLSEGIREWWALKPGAPQPKANQQHQDNARGLVLPGYKYLGPGNGLDKGEPVNAADAAALEHDKAYDQQLKAGDNPYLKYNHADAEFQERLKEDTSFGGNLGRAVFQAKKRLLEPLGLVEEAAKTAPGKKRPVEQSPQEPDSSAGIGKSGAQPAKKRLNFGQTGDTESVPDPQPIGEPPAAPSGVGSLTMASGGGAPVADNNEGADGVGSSSGNWHCDSQWLGDRVITTSTRTWALPTYNNHLYKQISNSTSGGSSNDNAYFGYSTPWGYFDFNRFHCHFSPRDWQRLINNNWGFRPKRLNFKLFNIQVKEVTDNNGVKTIANNLTSTVQVFTDSDYQLPYVLGSAHEGCLPPFPADVFMIPQYGYLTLNDGSQAVGRSSFYCLEYFPSQMLRTGNNFQFSYEFENVPFHSSYAHSQSLDRLMNPLIDQYLYYLSKTINGSGQNQQTLKFSVAGPSNMAVQGRNYIPGPSYRQQRVSTTVTQNNNSEFAWPGASSWALNGRNSLMNPGPAMASHKEGEDRFFPLSGSLIFGKQGTGRDNVDADKVMITNEEEIKTTNPVATESYGQVATNHQGQRGNYSRGVDAQAAQTGWVQNQGILPGMVWQDRDVYLQGPIWAKIPHTDGNFHPSPLMGGFGMKHPPPQILIKNTPVPADPPTAFNKDKLNSFITQYSTGQVSVEIEWELQKENSKRWNPEIQYTSNYYKSNNVEFAVNTEGVYSEPRPIGTRYLTRNL

SEQ ID NO: 5 - protein, 747 aa, Artificial Sequence
  AAVrh10 with insert A6
MAADGYLPDWLEDNLSEGIREWWDLKPGAPKPKANQQKQDDGRGLVLPGYKYLGPFNGLDKGEPVNAADAAALEHDKAYDQQLKAGDNPYLRYNHADAEFQERLQEDTSFGGNLGRAVFQAKKRVLEPLGLVEEGAKTAPGKKRPVEPSPQRSPDSSTGIGKKGQQPAKKRLNFGQTGDSESVPDPQPIGEPPAGPSGLGSGTMAAGGGAPMADNNEGADGVGSSSGNWHCDSTWLGDRVITTSTRTWALPTYNNHLYKQISNGTSGGSTNDNTYFGYSTPWGYFDFNRFHCHFSPRDWQRLINNNWGFRPKRLNFKLFNIQVKEVTQNEGTKTIANNLTSTIQVFTDSEYQLPYVLGSAHQGCLPPFPADVFMIPQYGYLTLNNGSQAVGRSSFYCLEYFPSQMLRTGNNFEFSYQFEDVPFHSSYAHSQSLDRLMNPLIDQYLYYLSRTQSTGGTAGTQQLLFSQAGPNNMSAQAKNWLPGPCYRQQRVSTTLSQNNNSNFAWTGATKYHLNGRDSLVNPGVAMATHKDDEERFFPSSGVLMFGKQGAGKDNVDYSSVMLTSEEEIKTTNPVATEQYGVVADNLQGQRGNEARVREAQAAIVGAVNSQGALPGMVWQNRDVYLQGPIWAKIPHTDGNFHPSPLMGGFGLKHPPPQILIKNTPVPADPPTTFSQAKLASFITQYSTGQVSVEIEWELQKENSKRWNPEIQYTSNYYKSTNVDFAVNTDGTYSEPRPIGTRYLTRNL

SEQ ID NO: 6 - protein, 747 aa, Artificial Sequence
  AAVrh10 with insert A2
MAADGYLPDWLEDNLSEGIREWWDLKPGAPKPKANQQKQDDGRGLVLPGYKYLGPFNGLDKGEPVNAADAAALEHDKAYDQQLKAGDNPYLRYNHADAEFQERLQEDTSFGGNLGRAVFQAKKRVLEPLGLVEEGAKTAPGKKRPVEPSPQRSPDSSTGIGKKGQQPAKKRLNFGQTGDSESVPDPQPIGEPPAGPSGLGSGTMAAGGGAPMADNNEGADGVGSSSGNWHCDSTWLGDRVITTSTRTWALPTYNNHLYKQISNGTSGGSTNDNTYFGYSTPWGYFDFNRFHCHFSPRDWQRLINNNWGFRPKRLNFKLFNIQVKEVTQNEGTKTIANNLTSTIQVFTDSEYQLPYVLGSAHQGCLPPFPADVFMIPQYGYLTLNNGSQAVGRSSFYCLEYFPSQMLRTGNNFEFSYQFEDVPFHSSYAHSQSLDRLMNPLIDQYLYYLSRTQSTGGTAGTQQLLFSQAGPNNMSAQAKNWLPGPCYRQQRVSTTLSQNNNSNFAWTGATKYHLNGRDSLVNPGVAMATHKDDEERFFPSSGVLMFGKQGAGKDNVDYSSVMLTSEEEIKTTNPVATEQYGVVADNLQGQRGNYSRGVDAQAAIVGAVNSQGALPGMVWQNRDVYLQGPIWAKIPHTDGNFHPSPLMGGFGLKHPPPQILIKNTPVPADPPTTFSQAKLASFITQYSTGQVSVEIEWELQKENSKRWNPEIQYTSNYYKSTNVDFAVNTDGTYSEPRPIGTRYLTRNL

SEQ ID NO: 7 - protein, 748 aa, Artificial Sequence
  AAVDJ with insert QR-P2
MAADGYLPDWLEDTLSEGIRQWWKLKPGPPPPKPAERHKDDSRGLVLPGYKYLGPFNGLDKGEPVNEADAAALEHDKAYDRQLDSGDNPYLKYNHADAEFQERLKEDTSFGGNLGRAVFQAKKRLLEPLGLVEEAAKTAPGKKRPVEHSPVEPDSSSGTGKAGQQPARKRLNFGQTGDADSVPDPQPIGEPPAAPSGVGSLTMAAGGGAPMADNNEGADGVGNSSGNWHCDSTWMGDRVITTSTRTWALPTYNNHLYKQISNSTSGGSSNDNAYFGYSTPWGYFDFNRFHCHFSPRDWQRLINNNWGFRPKRLSFKLFNIQVKEVTQNEGTKTIANNLTSTIQVFTDSEYQLPYVLGSAHQGCLPPFPADVFMIPQYGYLTLNNGSQAVGRSSFYCLEYFPSQMLRTGNNFQFTYTFEDVPFHSSYAHSQSLDRLMNPLIDQYLYYLSRTQTTGGTTNTQTLGFSQGGPNTMANQAKNWLPGPCYRQQRVSKTSADNNNSEYSWTGATKYHLNGRDSLVNPGPAMASHKDDEEKFFPQSGVLIFGKQGSEKTNVDIEKVMITDEEEIRTTNPVATEQYGSVSTNLQQGQRGCDCRGDCFCAQAATADVNTQGVLPGMVWQDRDVYLQGPIWAKIPHTDGHFHPSPLMGGFGLKHPPPQILIKNTPVPADPPTTFNQSKLNSFITQYSTGQVSVEIEWELQKENSKRWNPEIQYTSNYYKSTSVDFAVNTEGVYSEPRPIGTRYLTRNL

SEQ ID NO: 8 - protein, 15 aa, Artificial Sequence
  insert A2
GQRGNYSRGVDAQAA

SEQ ID NO: 9 - protein, 15 aa, Artificial Sequence
  insert A6
GQRGNEARVREAQAA

SEQ ID NO: 10 - protein, 18 aa, Artificial Sequence
  insert P2
QGQSGCDCRGDCFCAQAA

SEQ ID NO: 11 - protein, 15 aa, Artificial Sequence
  insert P4
GQSGNDVRSANAQAA

SEQ ID NO: 12 - protein, 18 aa, Artificial Sequence
  insert QR-P2
QGQRGCDCRGDCFCAQAA

SEQ ID NO: 13 - protein, 736 aa, adeno-associated virus 1
MAADGYLPDWLEDNLSEGIREWWDLKPGAPKPKANQQKQDDGRGLVLPGYKYLGPFNGLDKGEPVNAADAAALEHDKAYDQQLKAGDNPYLRYNHADAEFQERLQEDTSFGGNLGRAVFQAKKRVLEPLGLVEEGAKTAPGKKRPVEQSPQEPDSSSGIGKTGQQPAKKRLNFGQTGDSESVPDPQPLGEPPATPAAVGPTTMASGGGAPMADNNEGADGVGNASGNWHCDSTWLGDRVITTSTRTWALPTYNNHLYKQISSASTGASNDNHYFGYSTPWGYFDFNRFHCHFSPRDWQRLINNNWGFRPKRLNFKLFNIQVKEVTTNDGVTTIANNLTSTVQVFSDSEYQLPYVLGSAHQGCLPPFPADVFMIPQYGYLTLNNGSQAVGRSSFYCLEYFPSQMLRTGNNFTFSYTFEEVPFHSSYAHSQSLDRLMNPLIDQYLYYLNRTQNQSGSAQNKDLLFSRGSPAGMSVQPKNWLPGPCYRQQRVSKTKTDNNNSNFTWTGASKYNLNGRESIINPGTAMASHKDDEDKFFPMSGVMIFGKESAGASNTALDNVMITDEEEIKATNPVATERFGTVAVNFQSSSTDPATGDVHAMGALPGMVWQDRDVYLQGPIWAKIPHTDGHFHPSPLMGGFGLKNPPPQILIKNTPVPANPPAEFSATKFASFITQYSTGQVSVEIEWELQKENSKRWNPEVQYTSNYAKSANVDFTVDNNGLYTEPRPIGTRYLTRPL

SEQ ID NO: 14 - protein, 735 aa, adeno-associated virus 2 [sequence omitted]

SEQ ID NO: 15 - protein, 737 aa, adeno-associated virus 7
MAADGYLPDWLEDNLSEGIREWWDLKPGAPKPKANQQKQDNGRGLVLPGYKYLGPFNGLDKGEPVNAADAAALEHDKAYDQQLKAGDNPYLRYNHADAEFQERLQEDTSFGGNLGRAVFQAKKRVLEPLGLVEEGAKTAPAKKRPVEPSPQRSPDSSTGIGKKGQQPARKRLNFGQTGDSESVPDPQPLGEPPAAPSSVGSGTVAAGGGAPMADNNEGADGVGNASGNWHCDSTWLGDRVITTSTRTWALPTYNNHLYKQISSETAGSTNDNTYFGYSTPWGYFDFNRFHCHFSPRDWQRLINNNWGFRPKKLRFKLFNIQVKEVTTNDGVTTIANNLTSTIQVFSDSEYQLPYVLGSAHQGCLPPFPADVFMIPQYGYLTLNNGSQSVGRSSFYCLEYFPSQMLRTGNNFEFSYSFEDVPFHSSYAHSQSLDRLMNPLIDQYLYYLARTQSNPGGTAGNRELQFYQGGPSTMAEQAKNWLPGPCFRQQRVSKTLDQNNNSNFAWTGATKYHLNGRNSLVNPGVAMATHKDDEDRFFPSSGVLIFGKTGATNKTTLENVLMTNEEEIRPTNPVATEEYGIVSSNLQAANTAAQTQVVNNQGALPGMVWQNRDVYLQGPIWAKIPHTDGNFHPSPLMGGFGLKHPPPQILIKNTPVPANPPEVFTPAKFASFITQYSTGQVSVEIEWELQKENSKRWNPEIQYTSNFEKQTGVDFAVDSQGVYSEPRPIGTRYLTRNL

SEQ ID NO: 16 - protein, 736 aa, adeno-associated virus 9
MAADGYLPDWLEDNLSEGIREWWALKPGAPQPKANQQHQDNARGLVLPGYKYLGPGNGLDKGEPVNAADAAALEHDKAYDQQLKAGDNPYLKYNHADAEFQERLKEDTSFGGNLGRAVFQAKKRLLEPLGLVEEAAKTAPGKKRPVEQSPQEPDSSAGIGKSGAQPAKKRLNFGQTGDTESVPDPQPIGEPPAAPSGVGSLTMASGGGAPVADNNEGADGVGSSSGNWHCDSQWLGDRVITTSTRTWALPTYNNHLYKQISNSTSGGSSNDNAYFGYSTPWGYFDFNRFHCHFSPRDWQRLINNNWGFRPKRLNFKLFNIQVKEVTDNNGVKTIANNLTSTVQVFTDSDYQLPYVLGSAHEGCLPPFPADVFMIPQYGYLTLNDGSQAVGRSSFYCLEYFPSQMLRTGNNFQFSYEFENVPFHSSYAHSQSLDRLMNPLIDQYLYYLSKTINGSGQNQQTLKFSVAGPSNMAVQGRNYIPGPSYRQQRVSTTVTQNNNSEFAWPGASSWALNGRNSLMNPGPAMASHKEGEDRFFPLSGSLIFGKQGTGRDNVDADKVMITNEEEIKTTNPVATESYGQVATNHQSAQAQAQTGWVQNQGILPGMVWQDRDVYLQGPIWAKIPHTDGNFHPSPLMGGFGMKHPPPQILIKNTPVPADPPTAFNKDKLNSFITQYSTGQVSVEIEWELQKENSKRWNPEIQYTSNYYKSNNVEFAVNTEGVYSEPRPIGTRYLTRNL

SEQ ID NO: 17 - protein, 738 aa, adeno-associated virus rh10
MAADGYLPDWLEDNLSEGIREWWDLKPGAPKPKANQQKQDDGRGLVLPGYKYLGPFNGLDKGEPVNAADAAALEHDKAYDQQLKAGDNPYLRYNHADAEFQERLQEDTSFGGNLGRAVFQAKKRVLEPLGLVEEGAKTAPGKKRPVEPSPQRSPDSSTGIGKKGQQPAKKRLNFGQTGDSESVPDPQPIGEPPAGPSGLGSGTMAAGGGAPMADNNEGADGVGSSSGNWHCDSTWLGDRVITTSTRTWALPTYNNHLYKQISNGTSGGSTNDNTYFGYSTPWGYFDFNRFHCHFSPRDWQRLINNNWGFRPKRLNFKLFNIQVKEVTQNEGTKTIANNLTSTIQVFTDSEYQLPYVLGSAHQGCLPPFPADVFMIPQYGYLTLNNGSQAVGRSSFYCLEYFPSQMLRTGNNFEFSYQFEDVPFHSSYAHSQSLDRLMNPLIDQYLYYLSRTQSTGGTAGTQQLLFSQAGPNNMSAQAKNWLPGPCYRQQRVSTTLSQNNNSNFAWTGATKYHLNGRDSLVNPGVAMATHKDDEERFFPSSGVLMFGKQGAGKDNVDYSSVMLTSEEEIKTTNPVATEQYGVVADNLQQQNAAPIVGAVNSQGALPGMVWQNRDVYLQGPIWAKIPHTDGNFHPSPLMGGFGLKHPPPQILIKNTPVPADPPTTFSQAKLASFITQYSTGQVSVEIEWELQKENSKRWNPEIQYTSNYYKSTNVDFAVNTDGTYSEPRPIGTRYLTRNL

SEQ ID NO: 18 - protein, 737 aa, Artificial Sequence
  AAV DJ-QR
MAADGYLPDWLEDTLSEGIRQWWKLKPGPPPPKPAERHKDDSRGLVLPGYKYLGPFNGLDKGEPVNEADAAALEHDKAYDRQLDSGDNPYLKYNHADAEFQERLKEDTSFGGNLGRAVFQAKKRLLEPLGLVEEAAKTAPGKKRPVEHSPVEPDSSSGTGKAGQQPARKRLNFGQTGDADSVPDPQPIGEPPAAPSGVGSLTMAAGGGAPMADNNEGADGVGNSSGNWHCDSTWMGDRVITTSTRTWALPTYNNHLYKQISNSTSGGSSNDNAYFGYSTPWGYFDFNRFHCHFSPRDWQRLINNNWGFRPKRLSFKLFNIQVKEVTQNEGTKTIANNLTSTIQVFTDSEYQLPYVLGSAHQGCLPPFPADVFMIPQYGYLTLNNGSQAVGRSSFYCLEYFPSQMLRTGNNFQFTYTFEDVPFHSSYAHSQSLDRLMNPLIDQYLYYLSRTQTTGGTTNTQTLGFSQGGPNTMANQAKNWLPGPCYRQQRVSKTSADNNNSEYSWTGATKYHLNGRDSLVNPGPAMASHKDDEEKFFPQSGVLIFGKQGSEKTNVDIEKVMITDEEEIRTTNPVATEQYGSVSTNLQRGNRQAATADVNTQGVLPGMVWQDRDVYLQGPIWAKIPHTDGHFHPSPLMGGFGLKHPPPQILIKNTPVPADPPTTFNQSKLNSFITQYSTGQVSVEIEWELQKENSKRWNPEIQYTSNYYKSTSVDFAVNTEGVYSEPRPIGTRYLTRNL

SEQ ID NO: 19 - protein, 724 aa, adeno-associated virus 5
MSFVDHPPDWLEEVGEGLREFLGLEAGPPKPKPNQQHQDQARGLVLPGYNYLGPGNGLDRGEPVNRADEVAREHDISYNEQLEAGDNPYLKYNHADAEFQEKLADDTSFGGNLGKAVFQAKKRVLEPFGLVEEGAKTAPTGKRIDDHFPKRKKARTEEDSKPSTSSDAEAGPSGSQQLQIPAQPASSLGADTMSAGGGGPLGDNNQGADGVGNASGDWHCDSTWMGDRVVTKSTRTWVLPSYNNHQYREIKSGSVDGSNANAYFGYSTPWGYFDFNRFHSHWSPRDWQRLINNYWGFRPRSLRVKIFNIQVKEVTVQDSTTTIANNLTSTVQVFTDDDYQLPYVVGNGTEGCLPAFPPQVFTLPQYGYATLNRDNTENPTERSSFFCLEYFPSKMLRTGNNFEFTYNFEEVPFHSSFAPSQNLFKLANPLVDQYLYRFVSTNNTGGVQFNKNLAGRYANTYKNWFPGPMGRTQGWNLGSGVNRASVSAFATTNRMELEGASYQVPPQPNGMTNNLQGSNTYALENTMIFNSQPANPGTTATYLEGNMLITSESETQPVNRVAYNVGGQMATNNQSSTTAPATGTYNLQEIVPGSVWMERDVYLQGPIWAKIPETGAHFHPSPAMGGFGLKHPPPMMLIKNTPVPGNITSFSDVPVSSFITQYSTGQVTVEMEWELKKENSKRWNPEIQYTNNYNDPQFVDFAPDSTGEYRTTRPIGTRYLTRPL

SEQ ID NO: 20 - protein, 13 aa, Artificial Sequence
  insertAAV7A6
GQRGNEARVREAQ

SEQ ID NO: 21 - protein, 15 aa, Artificial Sequence
  insertAAV2P2
QGQSGCDCRGDCFCA

SEQ ID NO: 22 - protein, 15 aa, Artificial Sequence
  insertAAVDJQRP2
QGQRGCDCRGDCFCA

SEQ ID NO: 23 - protein, 17 aa, Artificial Sequence
  general formula I
  MISC_FEATURE (1)..(1): Xaa represents 0, 1 or 2 amino acid residues
  MISC_FEATURE (4)..(4): Xaa represents a single amino acid residue
  MISC_FEATURE (6)..(6): Xaa represents a single amino acid residue
  MISC_FEATURE (7)..(7): Xaa represents a single amino acid residue
  MISC_FEATURE (8)..(8): Xaa represents a single amino acid residue
  MISC_FEATURE (10)..(10): Xaa represents a single amino acid residue
  MISC_FEATURE (11)..(11): Xaa represents a single amino acid residue
  MISC_FEATURE (12)..(12): Xaa represents a single amino acid residue
  MISC_FEATURE (13)..(13): Xaa represents 0, 1 or 2 amino acid residues
XGQXGXXXRXXXXAQAA

SEQ ID NO: 24 - protein, 19 aa, Artificial Sequence
  alternative formula for sequence Z
  MISC_FEATURE (1)..(1): Xaa is Q or none
  MISC_FEATURE (4)..(4): Xaa is S or R
  MISC_FEATURE (6)..(6): Xaa is N or C
  MISC_FEATURE (7)..(7): Xaa is D, Y or E
  MISC_FEATURE (8)..(8): Xaa is C, V, S or A
  MISC_FEATURE (10)..(10): Xaa is G, S or V
  MISC_FEATURE (11)..(11): Xaa is none, A, V or R
  MISC_FEATURE (12)..(12): Xaa is D, N or E
  MISC_FEATURE (13)..(13): Xaa is  C or A
  MISC_FEATURE (14)..(14): Xaa is  F or Q
  MISC_FEATURE (15)..(15): Xaa is  none, C or A
  MISC_FEATURE (16)..(16): Xaa is  none or A
  MISC_FEATURE (17)..(17): Xaa is none or Q
  MISC_FEATURE (18)..(18): Xaa is none or A
  MISC_FEATURE (19)..(19): Xaa is none or A
XGQXGXXXRXXXXXXXXXX

SEQ ID NO: 25 - protein, 18 aa, Artificial Sequence
  alternative formula for sequence Z
  MISC_FEATURE (1)..(1): Xaa is Q or none
  MISC_FEATURE (4)..(4): Xaa is S or R
  MISC_FEATURE (6)..(6): Xaa is N or C
  MISC_FEATURE (7)..(7): Xaa is D, Y or E
  MISC_FEATURE (8)..(8): Xaa is C, V, S or A
  MISC_FEATURE (10)..(10): Xaa is G, S or V
  MISC_FEATURE (11)..(11): Xaa is none or D
  MISC_FEATURE (12)..(12): Xaa is none or C
  MISC_FEATURE (13)..(13): Xaa is A, V, R or F
  MISC_FEATURE (14)..(14): Xaa is N, D, E or C
  MISC_FEATURE (16)..(16): Xaa is none or Q
  MISC_FEATURE (17)..(17): Xaa is none or A
  MISC_FEATURE (18)..(18): Xaa is none or A
XGQXGXXXRXXXXXAXXX

SEQ ID NO: 26 - protein, 18 aa, Artificial Sequence
  preferred embodiment of formula I
  MISC_FEATURE (1)..(1): Xaa is none or Q
  MISC_FEATURE (4)..(4): Xaa is R or S
  MISC_FEATURE (6)..(6): Xaa is C or N
  MISC_FEATURE (7)..(7): Xaa is D, E or Y
  MISC_FEATURE (8)..(8): Xaa is C, A, S or V
  MISC_FEATURE (10)..(10): Xaa is G, V or S
  MISC_FEATURE (11)..(11): Xaa is D or none
  MISC_FEATURE (12)..(12): Xaa is C or none
  MISC_FEATURE (13)..(13): Xaa is F, R, V or A
  MISC_FEATURE (14)..(14): Xaa is C, D, N or E
XGQXGXXXRXXXXXAQAA

SEQ ID NO: 27 - protein, 52 aa, Artificial Sequence
  formula II
  MISC_FEATURE (5)..(8): Xaa represents a single amino acid residue
  MISC_FEATURE (14)..(15): Xaa represents a single amino acid residue
  MISC_FEATURE (17)..(20): Xaa represents a single amino acid residue
  MISC_FEATURE (22)..(22): Xaa represents a single amino acid residue
  MISC_FEATURE (24)..(24): Xaa represents 0, 1 or 2 amino acid residue(s)
  MISC_FEATURE (25)..(25): Xaa represents sequence Z
  MISC_FEATURE (26)..(26): Xaa represents 5, 6, 7, 8, 9, 10, 11, 12, 13, 14 or 15 amino acid residues
  MISC_FEATURE (34)..(34): Xaa represents a single amino acid residue
EEEIXXXXPVATEXXGXXXXNXQXXXLPGMVWQXRDVYLQGPIWAKIPHTDG